European Patent Specification EP 4 063 523 B1, published April 2, 2025. Title: Composition, Kit, Method for Detecting Sars-COV-2 and Use Thereof. Applicant: Sansure Biotech Inc. Application EP20939228.1. The sequence listing filed with the application follows.

SEQUENCE LISTING (48 sequences)

SEQ ID NO: 1 - DNA, 170 bp, SARS-CoV-2
acaattcacctaatttagcatggcctcttattgtaacagctttaagggccaattctgctgtcaaattacagaataatgagcttagtcctgttgcactacgacagatgtcttgtgctgccggtactacacaaactgcttgcactgatgacaatgcgttagcttactacaac

SEQ ID NO: 2 - DNA, 170 bp, SARS-CoV-2
actagaaggttctgttgcttatgaaagtttacgccctgacacacgttatgtgctcatggatggctctattattcaatttcctaacacctaccttgaaggttctgttagagtggtaacaacttttgattctgagtactgtaggcacggcacttgtgaaagatcagaagctg

SEQ ID NO: 3 - DNA, 152 bp, SARS-CoV-2
atggtatttctactacctaggaactgggccagaagctggacttccctatggtgctaacaaagacggcatcatatgggttgcaactgagggagccttgaatacaccaaaagatcacattggcacccgcaatcctgctaacaatgctgcaatcg

SEQ ID NO: 4 - DNA, 270 bp, Homo sapiens
gaattcggcacgaggtgggacttcagcatggcggtgtttgcagatttggacctgcgagcgggttctgacctgaaggctctgcgcggacttgtggagacagccgctcaccttggctattcagttgttgctatcaatcatatcgttgactttaaggaaaagaaacaggaaattgaaaaaccagtagctgtttctgaactcttcacaactttgccaattgtacagggaaaatcaagaccaattaaaattttaactagattaacaattattgtc

SEQ ID NO: 5 - DNA, 23 bp, Artificial Sequence
  Artificial Sequence
ggtatttctactacctaggaact

SEQ ID NO: 6 - DNA, 22 bp, Artificial Sequence
  Artificial Sequence
tgcagcattgttagcaggattg

SEQ ID NO: 7 - DNA, 27 bp, Artificial Sequence
  Artificial Sequence
gccagaagctggacttccctatggtgc

SEQ ID NO: 8 - DNA, 24 bp, Artificial Sequence
  Artificial Sequence
attcacctaatttagcatggcctc

SEQ ID NO: 9 - DNA, 24 bp, Artificial Sequence
  Artificial Sequence
acatctgtcgtagtgcaacaggac

SEQ ID NO: 10 - DNA, 31 bp, Artificial Sequence
  Artificial Sequence
ttgtaacagctttaagggccaattctgctgt

SEQ ID NO: 11 - DNA, 22 bp, Artificial Sequence
  Artificial Sequence
atggcctcttattgtaacagct

SEQ ID NO: 12 - DNA, 24 bp, Artificial Sequence
  Artificial Sequence
agcagtttgtgtagtaccggcagc

SEQ ID NO: 13 - DNA, 27 bp, Artificial Sequence
  Artificial Sequence
ccaattctgctgtcaaattacagaata

SEQ ID NO: 14 - DNA, 25 bp, Artificial Sequence
  Artificial Sequence
gaaggttctgttgcttatgaaagtt

SEQ ID NO: 15 - DNA, 21 bp, Artificial Sequence
  Artificial Sequence
taccactctaacagaaccttc

SEQ ID NO: 16 - DNA, 28 bp, Artificial Sequence
  Artificial Sequence
gccctgacacacgttatgtgctcatgga

SEQ ID NO: 17 - DNA, 20 bp, Artificial Sequence
  Artificial Sequence
atgaaagtttacgccctgac

SEQ ID NO: 18 - DNA, 23 bp, Artificial Sequence
  Artificial Sequence
ccgtgcctacagtactcagaatc

SEQ ID NO: 19 - DNA, 31 bp, Artificial Sequence
  Artificial Sequence
atgtgctcatggatggctctattattcaatt

SEQ ID NO: 20 - DNA, 21 bp, Artificial Sequence
  Artificial Sequence
gaggtgggacttcagcatggc

SEQ ID NO: 21 - DNA, 23 bp, Artificial Sequence
  Artificial Sequence
tgtttcttttccttaaagtcaac

SEQ ID NO: 22 - DNA, 27 bp, Artificial Sequence
  Artificial Sequence
agatttggacctgcgagcgggttctga

SEQ ID NO: 23 - DNA, 22 bp, Artificial Sequence
  Artificial Sequence
ggggaacttctcctgctagaat

SEQ ID NO: 24 - DNA, 22 bp, Artificial Sequence
  Artificial Sequence
cagacattttgctctcaagctg

SEQ ID NO: 25 - DNA, 20 bp, Artificial Sequence
  Artificial Sequence
ttgctgctgcttgacagatt

SEQ ID NO: 26 - DNA, 20 bp, Artificial Sequence
  Artificial Sequence
gaccccaaaatcagcgaaat

SEQ ID NO: 27 - DNA, 24 bp, Artificial Sequence
  Artificial Sequence
tctggttactgccagttgaatctg

SEQ ID NO: 28 - DNA, 24 bp, Artificial Sequence
  Artificial Sequence
accccgcattacgtttggtggacc

SEQ ID NO: 29 - DNA, 20 bp, Artificial Sequence
  Artificial Sequence
ttacaaacattggccgcaaa

SEQ ID NO: 30 - DNA, 18 bp, Artificial Sequence
  Artificial Sequence
gcgcgacattccgaagaa

SEQ ID NO: 31 - DNA, 23 bp, Artificial Sequence
  Artificial Sequence
acaatttgcccccagcgcttcag

SEQ ID NO: 32 - DNA, 22 bp, Artificial Sequence
  Artificial Sequence
gggagccttgaatacaccaaaa

SEQ ID NO: 33 - DNA, 21 bp, Artificial Sequence
  Artificial Sequence
tgtagcacgattgcagcattg

SEQ ID NO: 34 - DNA, 24 bp, Artificial Sequence
  Artificial Sequence
aycacattggcacccgcaatcctg

SEQ ID NO: 35 - DNA, 22 bp, Artificial Sequence
  Artificial Sequence
taatcagacaaggaactgatta

SEQ ID NO: 36 - DNA, 19 bp, Artificial Sequence
  Artificial Sequence
cgaaggtgtgacttccatg

SEQ ID NO: 37 - DNA, 20 bp, Artificial Sequence
  Artificial Sequence
gcaaattgtgcaatttgcgg

SEQ ID NO: 38 - DNA, 193 bp, SARS-CoV-2
ataaagaaatgtatctaaagttgcgtagtgatgtgctattacctcttacgcaatataatagatacttagctctttataataagtacaagtattttagtggagcaatggatacaactagctacagagaagctgcttgttgtcatctcgcaaaggctctcaatgacttcagtaactcaggttctgatgttcttta

SEQ ID NO: 39 - DNA, 20 bp, Artificial Sequence
  Artificial Sequence
atgtatctaaagttgcgtag

SEQ ID NO: 40 - DNA, 23 bp, Artificial Sequence
  Artificial Sequence
gttactgaagtcattgagagcct

SEQ ID NO: 41 - DNA, 29 bp, Artificial Sequence
  Artificial Sequence
atgtgctattacctcttacgcaatataat

SEQ ID NO: 42 - DNA, 219 bp, SARS-CoV-2
tgagagcaaaatgtctggtaaaggccaacaacaacaaggccaaactgtcactaagaaatctgctgctgaggcttctaagaagcctcggcaaaaacgtactgccactaaagcatacaatgtaacacaagctttcggcagacgtggtccagaacaaacccaaggaaattttggggaccaggaactaatcagacaaggaactgattacaaacattggccgca

SEQ ID NO: 43 - DNA, 21 bp, Artificial Sequence
  Artificial Sequence
actacctaggaactgggccag

SEQ ID NO: 44 - DNA, 21 bp, Artificial Sequence
  Artificial Sequence
agcaggattgcgggtgccaat

SEQ ID NO: 45 - DNA, 30 bp, Artificial Sequence
  Artificial Sequence
acttccctatggtgctaacaaagacggcat

SEQ ID NO: 46 - DNA, 22 bp, Artificial Sequence
  Artificial Sequence
atgtctggtaaaggccaacaac

SEQ ID NO: 47 - DNA, 21 bp, Artificial Sequence
  Artificial Sequence
agttccttgtctgattagttc

SEQ ID NO: 48 - DNA, 29 bp, Artificial Sequence
  Artificial Sequence
actgtcactaagaaatctgctgctgaggc